European Patent Application EP 4 276 197 A2, published November 15, 2023. Title: Mapping the Location, Type and Strand of Damaged and/or Mismatched Nucleotides in Double-Stranded DNA. Applicant: NEW ENGLAND BIOLABS, INC. Application EP. The sequence listing filed with the application follows.

SEQUENCE LISTING (1 sequence)

SEQ ID NO: 1 - DNA, 88 bp, synthetic construct
  misc_feature 1..88: note = Synthetic construct
  source 1..88: mol_type = other DNA
gagtcgatcgaatcgatcgatcgatcgatcgatcgatcgatgatctcagctagcttagctagctagctagctagctagctagctacta